European Patent Application EP 4 502 166 A1, published February 5, 2025. Title: Efficient production system for adeno-associated virus (AAV) vector. Applicant: 学校法人自治医科大学. The sequence listing filed with the application follows.

SEQUENCE LISTING (32 sequences)

SEQ ID NO: 1-3 - skipped (3 entries)

SEQ ID NO: 4 - DNA, 22 bp, synthetic construct
  misc_feature 1..22: note = 2xYY1 sequence
  source 1..22: mol_type = other DNA
ctccattttgagtctccatttt

SEQ ID NO: 5 - DNA, 48 bp, synthetic construct
  misc_feature 1..48: note = 4xYY1 sequence
  source 1..48: mol_type = other DNA
ctccattttgagtctccattttgagtctccattttgagtctccatttt

SEQ ID NO: 6 - DNA, 42 bp, synthetic construct
  misc_feature 1..42: note = InsYY1+1 sense
  source 1..42: mol_type = other DNA
tctccattttgaagcggggctagcatctgcgcagccgccatg

SEQ ID NO: 7 - DNA, 35 bp, synthetic construct
  misc_feature 1..35: note = InsYY1+1 Anti-sense
  source 1..35: mol_type = other DNA
ccctgcgagatctcttccgggggatccactagttc

SEQ ID NO: 8 - DNA, 30 bp, synthetic construct
  misc_feature 1..30: note = 2xYY1+1 sense
  source 1..30: mol_type = other DNA
aacgtctccattttgagtctccattttgat

SEQ ID NO: 9 - DNA, 34 bp, synthetic construct
  misc_feature 1..34: note = 2xYY1+1 Anti-sense
  source 1..34: mol_type = other DNA
ctagatcaaaatggagactcaaaatggagacgtt

SEQ ID NO: 10 - DNA, 56 bp, synthetic construct
  misc_feature 1..56: note = 4xYY1+1 sense
  source 1..56: mol_type = other DNA
aacgtctccattttgagtctccattttgagtctccattttgagtctccattttgat

SEQ ID NO: 11 - DNA, 60 bp, synthetic construct
  misc_feature 1..60: note = 4xYY1+1 Anti-sense
  source 1..60: mol_type = other DNA
ctagatcaaaatggagactcaaaatggagactcaaaatggagactcaaaatggagacgtt

SEQ ID NO: 12 - DNA, 21 bp, synthetic construct
  misc_feature 1..21: note = AAV2-ITR-qPCR-F
  source 1..21: mol_type = other DNA
ggaacccctagtgatggagtt

SEQ ID NO: 13 - DNA, 16 bp, synthetic construct
  misc_feature 1..16: note = AAV2-ITR-qPCR-R
  source 1..16: mol_type = other DNA
cggcctcagtgagcga

SEQ ID NO: 14 - DNA, 41 bp, synthetic construct
  misc_feature 1..41: note = AAV2-preRep-5p
  source 1..41: mol_type = other DNA
actagctagcaccggtcaattgatctgcgcagccgccatgc

SEQ ID NO: 15 - DNA, 47 bp, synthetic construct
  misc_feature 1..47: note = AAV2-preRep-3p
  source 1..47: mol_type = other DNA
cggaagatcttctagagatatctgagcttccaccactgtcttattcc

SEQ ID NO: 16 - DNA, 41 bp, synthetic construct
  misc_feature 1..41: note = AAV2-preCap-5p
  source 1..41: mol_type = other DNA
actagctagcaccggtcaattgagttgcgcagccatcgacg

SEQ ID NO: 17 - DNA, 48 bp, synthetic construct
  misc_feature 1..48: note = AAV2-preCap-3p
  source 1..48: mol_type = other DNA
cggaggatcctctagagatatcgcagagaccaaagttcaactgaaacg

SEQ ID NO: 18 - DNA, 41 bp, synthetic construct
  misc_feature 1..41: note = AAV2-Rep52-KZ-5p
  source 1..41: mol_type = other DNA
accgctcgaggctagcgccaccatggagctggtcgggtggc

SEQ ID NO: 19 - DNA, 41 bp, synthetic construct
  misc_feature 1..41: note = AAV2-Rep52-Stop-3p
  source 1..41: mol_type = other DNA
accgctcgagttattgttcaaagatgcagtcatccaaatcc

SEQ ID NO: 20 - DNA, 45 bp, synthetic construct
  misc_feature 1..45: note = AAV2-Rep78-KZ-5p
  source 1..45: mol_type = other DNA
actagctagccaattgccaccatgccggggttttacgagattgtg

SEQ ID NO: 21 - DNA, 47 bp, synthetic construct
  misc_feature 1..47: note = AAV2-Rep78-Stop-3p
  source 1..47: mol_type = other DNA
accgctcgagtctagattattgttcaaagatgcagtcatccaaatcc

SEQ ID NO: 22 - DNA, 70 bp, synthetic construct
  misc_feature 1..70: note = EcoRV-P2A-MfeI-EcoRI sense
  source 1..70: mol_type = other DNA
atcgctactaacttcagcctgctgaagcaggctggagacgtggaggagaaccctggacctgcaattgccg

SEQ ID NO: 23 - DNA, 74 bp, synthetic construct
  misc_feature 1..74: note = EcoRV-P2A-MfeI-EcoRI Anti-sense
  source 1..74: mol_type = other DNA
aattcggcaattgcaggtccagggttctcctccacgtctccagcctgcttcagcaggctgaagttagtagcgat

SEQ ID NO: 24 - DNA, 37 bp, synthetic construct
  misc_feature 1..37: note = AAV2-Rep52-no-Stop-3p
  source 1..37: mol_type = other DNA
ccggatatcttgttcaaagatgcagtcatccaaatcc

SEQ ID NO: 25 - DNA, 31 bp, synthetic construct
  misc_feature 1..31: note = AAV1,2,6,7,8,9,rh10-Cap-SwaI-5p
  source 1..31: mol_type = other DNA
aaatcaggtatggctgccgatggttatcttc

SEQ ID NO: 26 - DNA, 17 bp, synthetic construct
  misc_feature 1..17: note = M13-For
  source 1..17: mol_type = other DNA
gtaaaacgacggccagt

SEQ ID NO: 27 - DNA, 21 bp, synthetic construct
  misc_feature 1..21: note = AAV2,5,7,8,9,rh10 Cap-PmeI-3p
  source 1..21: mol_type = other DNA
cgcaaaacactcacgtgacct

SEQ ID NO: 28 - DNA, 33 bp, synthetic construct
  misc_feature 1..33: note = AAV1 Cap1 -XbaI-XmaI-3p
  source 1..33: mol_type = other DNA
tccccccgggcctctagaactagtggatccccc

SEQ ID NO: 29 - DNA, 31 bp, synthetic construct
  misc_feature 1..31: note = AAV1 Cap1 -EcoRV-3p-2
  source 1..31: mol_type = other DNA
ccggatatcgcgcaaccaagcagttaatgtg

SEQ ID NO: 30 - DNA, 30 bp, synthetic construct
  misc_feature 1..30: note = AAV7,8,9,rh10 preCap-EcoRV-3p
  source 1..30: mol_type = other DNA
ccggatatccaggacctctagtcctgcagg

SEQ ID NO: 31 - DNA, 41 bp, synthetic construct
  misc_feature 1..41: note = AAV9.47,PHP.eB,S Cap-SawI-5p
  source 1..41: mol_type = other DNA
acgatgatttaaatcaggtatggctgccgatggttatcttc

SEQ ID NO: 32 - DNA, 30 bp, synthetic construct
  misc_feature 1..30: note = AAV9.47,PHP.eB,S Cap-XmaI-3p
  source 1..30: mol_type = other DNA
tccccccggggcccttcgcagagaccaaag